European Patent Specification EP 3 250 691 B1, published June 21, 2023. Title: CRISPR HYBRID DNA/RNA POLYNUCLEOTIDES AND METHODS OF USE. Applicant: PIONEER HI-BRED INTERNATIONAL, INC. The sequence listing filed with the application follows.

SEQUENCE LISTING (254 sequences)

SEQ ID NO: 1 - RNA, 121 nt, Artificial Sequence
  source: /note="Description of Artificial Sequence: Synthetic polynucleotide"
ggggccacuagggacaggaugucucagagcuaugcuguccuggaaacaggacagcauagcaaguugagauaaggcuaguccguuaucaacuugaaaaaguggcaccgagucggugcuuuuu

SEQ ID NO: 2 - RNA, 73 nt, Artificial Sequence
  source: /note="Description of Artificial Sequence: Synthetic oligonucleotide"
gcaggacagcauagcaaguugagauaaggcuaguccguuaucaacuugaaaaaguggcaccgagucggugcuu

SEQ ID NO: 3 - DNA, 42 bp, Artificial Sequence
  source: /note="Description of Artificial Sequence: Synthetic oligonucleotide"
gagtccgagcagaagaagaagtctcagagctatgctgtcctg

SEQ ID NO: 4 - DNA, 42 bp, Artificial Sequence
  source: /note="Description of Artificial Sequence: Synthetic oligonucleotide"
gggtggggggagtttgctccgtctcagagctatgctgtcctg

SEQ ID NO: 5 - DNA, 42 bp, Artificial Sequence
  source: /note="Description of Artificial Sequence: Synthetic oligonucleotide"
gtttgtgtttccataaactggtctcagagctatgctgtcctg

SEQ ID NO: 6 - DNA, 42 bp, Artificial Sequence
  source: /note="Description of Artificial Sequence: Synthetic oligonucleotide"
tctgtgataacctcagtttagtctcagagctatgctgtcctg

SEQ ID NO: 7 - DNA, 42 bp, Artificial Sequence
  source: /note="Description of Artificial Sequence: Synthetic oligonucleotide"
ggccactgtagtcctccagggtctcagagctatgctgtcctg

SEQ ID NO: 8 - DNA, 42 bp, Artificial Sequence
  source: /note="Description of Artificial Sequence: Synthetic oligonucleotide"
gtcccccagccggtcagccagtctcagagctatgctgtcctg

SEQ ID NO: 9 - DNA, 42 bp, Artificial Sequence
  source: /note="Description of Artificial Sequence: Synthetic oligonucleotide"
ggcagccagcatgatgagacgtctcagagctatgctgtcctg

SEQ ID NO: 10 - DNA, 42 bp, Artificial Sequence
  source: /note="Description of Artificial Sequence: Synthetic oligonucleotide"
gaggagctccaagaagactggtctcagagctatgctgtcctg

SEQ ID NO: 11 - RNA, 42 nt, Artificial Sequence
  source: /note="Description of Artificial Sequence: Synthetic oligonucleotide"
gaguccgagcagaagaagaagucucagagcuaugcuguccug

SEQ ID NO: 12 - RNA, 42 nt, Artificial Sequence
  source: /note="Description of Artificial Sequence: Synthetic oligonucleotide"
ggguggggggaguuugcuccgucucagagcuaugcuguccug

SEQ ID NO: 13 - RNA, 42 nt, Artificial Sequence
  source: /note="Description of Artificial Sequence: Synthetic oligonucleotide"
guuuguguuuccauaaacuggucucagagcuaugcuguccug

SEQ ID NO: 14 - RNA, 42 nt, Artificial Sequence
  source: /note="Description of Artificial Sequence: Synthetic oligonucleotide"
ucugugauaaccucaguuuagucucagagcuaugcuguccug

SEQ ID NO: 15 - RNA, 42 nt, Artificial Sequence
  source: /note="Description of Artificial Sequence: Synthetic oligonucleotide"
ggccacuguaguccuccagggucucagagcuaugcuguccug

SEQ ID NO: 16 - RNA, 42 nt, Artificial Sequence
  source: /note="Description of Artificial Sequence: Synthetic oligonucleotide"
gucccccagccggucagccagucucagagcuaugcuguccug

SEQ ID NO: 17 - RNA, 42 nt, Artificial Sequence
  source: /note="Description of Artificial Sequence: Synthetic oligonucleotide"
ggcagccagcaugaugagacgucucagagcuaugcuguccug

SEQ ID NO: 18 - RNA, 42 nt, Artificial Sequence
  source: /note="Description of Artificial Sequence: Synthetic oligonucleotide"
gaggagcuccaagaagacuggucucagagcuaugcuguccug

SEQ ID NO: 19 - DNA, 42 bp, Artificial Sequence
  source: /note="Description of Artificial Sequence: Synthetic oligonucleotide"
  source: /note="Description of Combined DNA/RNA Molecule: Synthetic oligonucleotide"
gagtccgagcagaagaagaagucucagagctatgctgtcctg

SEQ ID NO: 20 - DNA, 42 bp, Artificial Sequence
  source: /note="Description of Artificial Sequence: Synthetic oligonucleotide"
  source: /note="Description of Combined DNA/RNA Molecule: Synthetic oligonucleotide"
gggtggggggagttugcuccgucucagagctatgctgtcctg

SEQ ID NO: 21 - DNA, 42 bp, Artificial Sequence
  source: /note="Description of Artificial Sequence: Synthetic oligonucleotide"
  source: /note="Description of Combined DNA/RNA Molecule: Synthetic oligonucleotide"
gtttgtgtttccataaacuggucucagagctatgctgtcctg

SEQ ID NO: 22 - DNA, 42 bp, Artificial Sequence
  source: /note="Description of Artificial Sequence: Synthetic oligonucleotide"
  source: /note="Description of Combined DNA/RNA Molecule: Synthetic oligonucleotide"
tctgtgataacctcaguuuagucucagagctatgctgtcctg

SEQ ID NO: 23 - DNA, 42 bp, Artificial Sequence
  source: /note="Description of Artificial Sequence: Synthetic oligonucleotide"
  source: /note="Description of Combined DNA/RNA Molecule: Synthetic oligonucleotide"
ggccactgtagtccuccagggucucagagctatgctgtcctg

SEQ ID NO: 24 - DNA, 42 bp, Artificial Sequence
  source: /note="Description of Artificial Sequence: Synthetic oligonucleotide"
  source: /note="Description of Combined DNA/RNA Molecule: Synthetic oligonucleotide"
gtcccccagccggtcagccagucucagagctatgctgtcctg

SEQ ID NO: 25 - DNA, 42 bp, Artificial Sequence
  source: /note="Description of Artificial Sequence: Synthetic oligonucleotide"
  source: /note="Description of Combined DNA/RNA Molecule: Synthetic oligonucleotide"
ggcagccagcatgaugagacgucucagagctatgctgtcctg

SEQ ID NO: 26 - DNA, 42 bp, Artificial Sequence
  source: /note="Description of Artificial Sequence: Synthetic oligonucleotide"
  source: /note="Description of Combined DNA/RNA Molecule: Synthetic oligonucleotide"
gaggagctccaagaagacuggucucagagctatgctgtcctg

SEQ ID NO: 27 - DNA, 20 bp, Homo sapiens
gagtccgagcagaagaagaa

SEQ ID NO: 28 - DNA, 20 bp, Homo sapiens
gagttagagcagaagaagaa

SEQ ID NO: 29 - DNA, 20 bp, Homo sapiens
aggtactagcagaagaagaa

SEQ ID NO: 30 - DNA, 20 bp, Homo sapiens
acgtctgagcagaagaagaa

SEQ ID NO: 31 - DNA, 20 bp, Homo sapiens
aggtgctagcagaagaagaa

SEQ ID NO: 32 - DNA, 20 bp, Homo sapiens
gggtggggggagtttgctcc

SEQ ID NO: 33 - DNA, 20 bp, Homo sapiens
ggatggagggagtttgctcc

SEQ ID NO: 34 - DNA, 20 bp, Homo sapiens
ggggaggggaagtttgctcc

SEQ ID NO: 35 - DNA, 20 bp, Homo sapiens
gggagggtggagtttgctcc

SEQ ID NO: 36 - DNA, 20 bp, Homo sapiens
cgggggagggagtttgctcc

SEQ ID NO: 37 - DNA, 42 bp, Artificial Sequence
  source: /note="Description of Artificial Sequence: Synthetic oligonucleotide"
ggggccactagggacaggatgtctcagagctatgctgtcctg

SEQ ID NO: 38 - DNA, 42 bp, Artificial Sequence
  source: /note="Description of Artificial Sequence: Synthetic oligonucleotide"
  source: /note="Description of Combined DNA/RNA Molecule: Synthetic oligonucleotide"
ggggccactagggacaggatgucucagagctatgctgtcctg

SEQ ID NO: 39 - DNA, 42 bp, Artificial Sequence; identical to SEQ ID NO: 37
  source: /note="Description of Artificial Sequence: Synthetic oligonucleotide"
  source: /note="Description of Combined DNA/RNA Molecule: Synthetic oligonucleotide"

SEQ ID NO: 40 - DNA, 42 bp, Artificial Sequence
  source: /note="Description of Artificial Sequence: Synthetic oligonucleotide"
  source: /note="Description of Combined DNA/RNA Molecule: Synthetic oligonucleotide"
ggggccactagggacaggaugtctcagagctatgctgtcctg

SEQ ID NO: 41 - DNA, 42 bp, Artificial Sequence
  source: /note="Description of Artificial Sequence: Synthetic oligonucleotide"
  source: /note="Description of Combined DNA/RNA Molecule: Synthetic oligonucleotide"
ggggccactagggacaggaugucucagagctatgctgtcctg

SEQ ID NO: 42 - DNA, 42 bp, Artificial Sequence
  source: /note="Description of Artificial Sequence: Synthetic oligonucleotide"
  source: /note="Description of Combined DNA/RNA Molecule: Synthetic oligonucleotide"
ggggccacuagggacaggaugtctcagagctatgctgtcctg

SEQ ID NO: 43 - DNA, 42 bp, Artificial Sequence; identical to SEQ ID NO: 38
  source: /note="Description of Artificial Sequence: Synthetic oligonucleotide"
  source: /note="Description of Combined DNA/RNA Molecule: Synthetic oligonucleotide"

SEQ ID NO: 44 - DNA, 42 bp, Artificial Sequence; identical to SEQ ID NO: 40
  source: /note="Description of Artificial Sequence: Synthetic oligonucleotide"
  source: /note="Description of Combined DNA/RNA Molecule: Synthetic oligonucleotide"

SEQ ID NO: 45 - DNA, 42 bp, Artificial Sequence; identical to SEQ ID NO: 38
  source: /note="Description of Artificial Sequence: Synthetic oligonucleotide"
  source: /note="Description of Combined DNA/RNA Molecule: Synthetic oligonucleotide"

SEQ ID NO: 46 - DNA, 42 bp, Artificial Sequence; identical to SEQ ID NO: 42
  source: /note="Description of Artificial Sequence: Synthetic oligonucleotide"
  source: /note="Description of Combined DNA/RNA Molecule: Synthetic oligonucleotide"

SEQ ID NO: 47 - DNA, 42 bp, Artificial Sequence
  source: /note="Description of Artificial Sequence: Synthetic oligonucleotide"
  source: /note="Description of Combined DNA/RNA Molecule: Synthetic oligonucleotide"
ggggccacuagggacaggatgucucagagctatgctgtcctg

SEQ ID NO: 48 - DNA, 42 bp, Artificial Sequence; identical to SEQ ID NO: 47
  source: /note="Description of Artificial Sequence: Synthetic oligonucleotide"
  source: /note="Description of Combined DNA/RNA Molecule: Synthetic oligonucleotide"

SEQ ID NO: 49 - DNA, 42 bp, Artificial Sequence
  source: /note="Description of Artificial Sequence: Synthetic oligonucleotide"
  source: /note="Description of Combined DNA/RNA Molecule: Synthetic oligonucleotide"
ggggccactagggacaggaugtcucagagctatgctgtcctg

SEQ ID NO: 50 - DNA, 42 bp, Artificial Sequence
  source: /note="Description of Artificial Sequence: Synthetic oligonucleotide"
  source: /note="Description of Combined DNA/RNA Molecule: Synthetic oligonucleotide"
ggggccactagggacaggauguctcagagctatgctgtcctg

SEQ ID NO: 51 - DNA, 42 bp, Artificial Sequence; identical to SEQ ID NO: 37
  source: /note="Description of Artificial Sequence: Synthetic oligonucleotide"
  source: /note="Description of Combined DNA/RNA Molecule: Synthetic oligonucleotide"

SEQ ID NO: 52 - DNA, 42 bp, Artificial Sequence; identical to SEQ ID NO: 40
  source: /note="Description of Artificial Sequence: Synthetic oligonucleotide"
  source: /note="Description of Combined DNA/RNA Molecule: Synthetic oligonucleotide"

SEQ ID NO: 53 - DNA, 42 bp, Artificial Sequence
  source: /note="Description of Artificial Sequence: Synthetic oligonucleotide"
  source: /note="Description of Combined DNA/RNA Molecule: Synthetic oligonucleotide"
ggggccactagggacaggatguctcagagctatgctgtcctg

SEQ ID NO: 54 - DNA, 42 bp, Artificial Sequence
  source: /note="Description of Artificial Sequence: Synthetic oligonucleotide"
  source: /note="Description of Combined DNA/RNA Molecule: Synthetic oligonucleotide"
ggggccactagggacaggatgtcucagagctatgctgtcctg

SEQ ID NO: 55 - DNA, 42 bp, Artificial Sequence; identical to SEQ ID NO: 37
  source: /note="Description of Artificial Sequence: Synthetic oligonucleotide"
  source: /note="Description of Combined DNA/RNA Molecule: Synthetic oligonucleotide"

SEQ ID NO: 56 - DNA, 42 bp, Artificial Sequence; identical to SEQ ID NO: 53
  source: /note="Description of Artificial Sequence: Synthetic oligonucleotide"
  source: /note="Description of Combined DNA/RNA Molecule: Synthetic oligonucleotide"

SEQ ID NO: 57 - DNA, 42 bp, Artificial Sequence; identical to SEQ ID NO: 54
  source: /note="Description of Artificial Sequence: Synthetic oligonucleotide"
  source: /note="Description of Combined DNA/RNA Molecule: Synthetic oligonucleotide"

SEQ ID NO: 58 - DNA, 42 bp, Artificial Sequence; identical to SEQ ID NO: 37
  source: /note="Description of Artificial Sequence: Synthetic oligonucleotide"
  source: /note="Description of Combined DNA/RNA Molecule: Synthetic oligonucleotide"

SEQ ID NO: 59 - DNA, 42 bp, Artificial Sequence; identical to SEQ ID NO: 37
  source: /note="Description of Artificial Sequence: Synthetic oligonucleotide"
  source: /note="Description of Combined DNA/RNA Molecule: Synthetic oligonucleotide"

SEQ ID NO: 60 - DNA, 42 bp, Artificial Sequence; identical to SEQ ID NO: 37
  source: /note="Description of Artificial Sequence: Synthetic oligonucleotide"

SEQ ID NO: 61 - DNA, 42 bp, Artificial Sequence; identical to SEQ ID NO: 37
  source: /note="Description of Artificial Sequence: Synthetic oligonucleotide"
  source: /note="Description of Combined DNA/RNA Molecule: Synthetic oligonucleotide"

SEQ ID NO: 62 - DNA, 42 bp, Artificial Sequence; identical to SEQ ID NO: 37
  source: /note="Description of Artificial Sequence: Synthetic oligonucleotide"
  source: /note="Description of Combined DNA/RNA Molecule: Synthetic oligonucleotide"

SEQ ID NO: 63 - DNA, 23 bp, Artificial Sequence
  source: /note="Description of Artificial Sequence: Synthetic oligonucleotide"
agtaataatacgactcactatag

SEQ ID NO: 64 - DNA, 58 bp, Artificial Sequence
  source: /note="Description of Artificial Sequence: Synthetic oligonucleotide"
taatacgactcactatagggggccactagggacaggatgttttagagctagaaatagc

SEQ ID NO: 65 - DNA, 50 bp, Artificial Sequence
  source: /note="Description of Artificial Sequence: Synthetic oligonucleotide"
gttttagagctagaaatagcaagttaaaataaggctagtccgttatcaac

SEQ ID NO: 66 - DNA, 50 bp, Artificial Sequence
  source: /note="Description of Artificial Sequence: Synthetic oligonucleotide"
aaaaaaagcaccgactcggtgccactttttcaagttgataacggactagc

SEQ ID NO: 67 - DNA, 23 bp, Artificial Sequence
  source: /note="Description of Artificial Sequence: Synthetic oligonucleotide"
aaaaaaagcaccgactcggtgcc

SEQ ID NO: 68 - DNA, 43 bp, Artificial Sequence
  source: /note="Description of Artificial Sequence: Synthetic oligonucleotide"
agtaataatacgactcactatagggggccactagggacaggat

SEQ ID NO: 69 - DNA, 42 bp, Artificial Sequence; identical to SEQ ID NO: 37
  source: /note="Description of Artificial Sequence: Synthetic oligonucleotide"

SEQ ID NO: 70 - DNA, 24 bp, Artificial Sequence
  source: /note="Description of Artificial Sequence: Synthetic oligonucleotide"
caggatgtctcagagctatgctgt

SEQ ID NO: 71 - DNA, 58 bp, Artificial Sequence
  source: /note="Description of Artificial Sequence: Synthetic oligonucleotide"
agtaataatacgactcactatagcaggacagcatagcaagttgagataaggctagtcc

SEQ ID NO: 72 - DNA, 42 bp, Artificial Sequence
  source: /note="Description of Artificial Sequence: Synthetic oligonucleotide"
gcaggacagcatagcaagttgagataaggctagtccgttatc

SEQ ID NO: 73 - DNA, 50 bp, Artificial Sequence
  source: /note="Description of Artificial Sequence: Synthetic oligonucleotide"
aagcaccgactcggtgccactttttcaagttgataacggactagccttat

SEQ ID NO: 74 - DNA, 20 bp, Artificial Sequence
  source: /note="Description of Artificial Sequence: Synthetic oligonucleotide"
aagcaccgactcggtgccac

SEQ ID NO: 75 - DNA, 20 bp, Artificial Sequence
  source: /note="Description of Artificial Sequence: Synthetic oligonucleotide"
ccccgttctcctgtggattc

SEQ ID NO: 76 - DNA, 20 bp, Artificial Sequence
  source: /note="Description of Artificial Sequence: Synthetic oligonucleotide"
atcctctctggctccatcgt

SEQ ID NO: 77 - DNA, 52 bp, Artificial Sequence
  source: /note="Description of Artificial Sequence: Synthetic oligonucleotide"
cactctttccctacacgacgctcttccgatctgtttctcatctgtgcccctc

SEQ ID NO: 78 - DNA, 48 bp, Artificial Sequence
  source: /note="Description of Artificial Sequence: Synthetic oligonucleotide"
ggagttcagacgtgtgctcttccgatctgttgcccaccctagtcattg

SEQ ID NO: 79 - DNA, 52 bp, Artificial Sequence
  source: /note="Description of Artificial Sequence: Synthetic oligonucleotide"
cactctttccctacacgacgctcttccgatctccagatggcacattgtcaga

SEQ ID NO: 80 - DNA, 47 bp, Artificial Sequence
  source: /note="Description of Artificial Sequence: Synthetic oligonucleotide"
ggagttcagacgtgtgctcttccgatctcctagtgactgccgtctgc

SEQ ID NO: 81 - DNA, 52 bp, Artificial Sequence
  source: /note="Description of Artificial Sequence: Synthetic oligonucleotide"
cactctttccctacacgacgctcttccgatctacatgcacacccatgttttg

SEQ ID NO: 82 - DNA, 48 bp, Artificial Sequence
  source: /note="Description of Artificial Sequence: Synthetic oligonucleotide"
ggagttcagacgtgtgctcttccgatctaacatttccaggtgacaggc

SEQ ID NO: 83 - DNA, 52 bp, Artificial Sequence; identical to SEQ ID NO: 81
  source: /note="Description of Artificial Sequence: Synthetic oligonucleotide"

SEQ ID NO: 84 - DNA, 48 bp, Artificial Sequence; identical to SEQ ID NO: 82
  source: /note="Description of Artificial Sequence: Synthetic oligonucleotide"

SEQ ID NO: 85 - DNA, 52 bp, Artificial Sequence
  source: /note="Description of Artificial Sequence: Synthetic oligonucleotide"
cactctttccctacacgacgctcttccgatctacatgaaattcaaggccgaa

SEQ ID NO: 86 - DNA, 48 bp, Artificial Sequence
  source: /note="Description of Artificial Sequence: Synthetic oligonucleotide"
ggagttcagacgtgtgctcttccgatctacctgtctgtgaggtggagg

SEQ ID NO: 87 - DNA, 52 bp, Artificial Sequence
  source: /note="Description of Artificial Sequence: Synthetic oligonucleotide"
cactctttccctacacgacgctcttccgatctgctggtggattatgggaatg

SEQ ID NO: 88 - DNA, 48 bp, Artificial Sequence
  source: /note="Description of Artificial Sequence: Synthetic oligonucleotide"
ggagttcagacgtgtgctcttccgatctagaagacctcatccttgggg

SEQ ID NO: 89 - DNA, 52 bp, Artificial Sequence
  source: /note="Description of Artificial Sequence: Synthetic oligonucleotide"
cactctttccctacacgacgctcttccgatctaagaaaggcaagaagcctgg

SEQ ID NO: 90 - DNA, 48 bp, Artificial Sequence
  source: /note="Description of Artificial Sequence: Synthetic oligonucleotide"
ggagttcagacgtgtgctcttccgatctgctggcctgagacattccta

SEQ ID NO: 91 - DNA, 52 bp, Artificial Sequence
  source: /note="Description of Artificial Sequence: Synthetic oligonucleotide"
cactctttccctacacgacgctcttccgatcttgtgtactctccactgccca

SEQ ID NO: 92 - DNA, 48 bp, Artificial Sequence
  source: /note="Description of Artificial Sequence: Synthetic oligonucleotide"
ggagttcagacgtgtgctcttccgatcttcagaacactcccttttgcc

SEQ ID NO: 93 - DNA, 52 bp, Artificial Sequence
  source: /note="Description of Artificial Sequence: Synthetic oligonucleotide"
cactctttccctacacgacgctcttccgatcttctggcaaggagagagatgg

SEQ ID NO: 94 - DNA, 48 bp, Artificial Sequence
  source: /note="Description of Artificial Sequence: Synthetic oligonucleotide"
ggagttcagacgtgtgctcttccgatcttatattcccagggccggtta

SEQ ID NO: 95 - DNA, 57 bp, Artificial Sequence
  source: /note="Description of Artificial Sequence: Synthetic oligonucleotide"
caagcagaagacggcatacgagattacgtgatgtgactggagttcagacgtgtgctc

SEQ ID NO: 96 - DNA, 57 bp, Artificial Sequence
  source: /note="Description of Artificial Sequence: Synthetic oligonucleotide"
caagcagaagacggcatacgagatattgccgagtgactggagttcagacgtgtgctc

SEQ ID NO: 97 - DNA, 57 bp, Artificial Sequence
  source: /note="Description of Artificial Sequence: Synthetic oligonucleotide"
caagcagaagacggcatacgagatattggtcagtgactggagttcagacgtgtgctc

SEQ ID NO: 98 - DNA, 57 bp, Artificial Sequence
  source: /note="Description of Artificial Sequence: Synthetic oligonucleotide"
caagcagaagacggcatacgagattaaaaatggtgactggagttcagacgtgtgctc

SEQ ID NO: 99 - DNA, 57 bp, Artificial Sequence
  source: /note="Description of Artificial Sequence: Synthetic oligonucleotide"
caagcagaagacggcatacgagatatcactgtgtgactggagttcagacgtgtgctc

SEQ ID NO: 100 - DNA, 57 bp, Artificial Sequence
  source: /note="Description of Artificial Sequence: Synthetic oligonucleotide"
caagcagaagacggcatacgagattatttcacgtgactggagttcagacgtgtgctc

SEQ ID NO: 101 - DNA, 58 bp, Artificial Sequence
  source: /note="Description of Artificial Sequence: Synthetic oligonucleotide"
aatgatacggcgaccaccgagatctacaccgtctaatacactctttccctacacgacg

SEQ ID NO: 102 - DNA, 58 bp, Artificial Sequence
  source: /note="Description of Artificial Sequence: Synthetic oligonucleotide"
aatgatacggcgaccaccgagatctacactctctccgacactctttccctacacgacg

SEQ ID NO: 103 - DNA, 58 bp, Artificial Sequence
  source: /note="Description of Artificial Sequence: Synthetic oligonucleotide"
aatgatacggcgaccaccgagatctacactcgactagacactctttccctacacgacg

SEQ ID NO: 104 - DNA, 58 bp, Artificial Sequence
  source: /note="Description of Artificial Sequence: Synthetic oligonucleotide"
aatgatacggcgaccaccgagatctacacttctagctacactctttccctacacgacg

SEQ ID NO: 105 - DNA, 58 bp, Artificial Sequence
  source: /note="Description of Artificial Sequence: Synthetic oligonucleotide"
aatgatacggcgaccaccgagatctacaccctagagtacactctttccctacacgacg

SEQ ID NO: 106 - DNA, 58 bp, Artificial Sequence
  source: /note="Description of Artificial Sequence: Synthetic oligonucleotide"
aatgatacggcgaccaccgagatctacacctattaagacactctttccctacacgacg

SEQ ID NO: 107 - DNA, 21 bp, Artificial Sequence
  source: /note="Description of Artificial Sequence: Synthetic oligonucleotide"
aaaaccacccttctctctggc

SEQ ID NO: 108 - DNA, 21 bp, Artificial Sequence
  source: /note="Description of Artificial Sequence: Synthetic oligonucleotide"
ggagattggagacacggagag

SEQ ID NO: 109 - DNA, 20 bp, Artificial Sequence
  source: /note="Description of Artificial Sequence: Synthetic oligonucleotide"
aaaggtgccttttgtgggga

SEQ ID NO: 110 - DNA, 21 bp, Artificial Sequence
  source: /note="Description of Artificial Sequence: Synthetic oligonucleotide"
acaatgggaaggacagcttct

SEQ ID NO: 111 - DNA, 20 bp, Artificial Sequence
  source: /note="Description of Artificial Sequence: Synthetic oligonucleotide"
tctccgaacttctgctgagc

SEQ ID NO: 112 - DNA, 20 bp, Artificial Sequence
  source: /note="Description of Artificial Sequence: Synthetic oligonucleotide"
tgactagcaaagcaggaggc

SEQ ID NO: 113 - DNA, 20 bp, Artificial Sequence
  source: /note="Description of Artificial Sequence: Synthetic oligonucleotide"
aagtccttcccatcgctgtg

SEQ ID NO: 114 - DNA, 20 bp, Artificial Sequence
  source: /note="Description of Artificial Sequence: Synthetic oligonucleotide"
gggaatgggaatgtgaggca

SEQ ID NO: 115 - DNA, 20 bp, Artificial Sequence
  source: /note="Description of Artificial Sequence: Synthetic oligonucleotide"
gagtccctgctctcctctga

SEQ ID NO: 116 - DNA, 20 bp, Artificial Sequence
  source: /note="Description of Artificial Sequence: Synthetic oligonucleotide"
agggaataccaaaacggcgt

SEQ ID NO: 117 - DNA, 20 bp, Artificial Sequence
  source: /note="Description of Artificial Sequence: Synthetic oligonucleotide"
gtcagagggacacactgtgg

SEQ ID NO: 118 - DNA, 20 bp, Artificial Sequence
  source: /note="Description of Artificial Sequence: Synthetic oligonucleotide"
aggagggagcaggaaagtga

SEQ ID NO: 119 - DNA, 20 bp, Artificial Sequence
  source: /note="Description of Artificial Sequence: Synthetic oligonucleotide"
ctcctgctccatgtgaccac

SEQ ID NO: 120 - DNA, 20 bp, Artificial Sequence
  source: /note="Description of Artificial Sequence: Synthetic oligonucleotide"
gtagtggcacagtcacagct

SEQ ID NO: 121 - DNA, 20 bp, Artificial Sequence
  source: /note="Description of Artificial Sequence: Synthetic oligonucleotide"
gagttgcagactggagctgt

SEQ ID NO: 122 - DNA, 20 bp, Artificial Sequence
  source: /note="Description of Artificial Sequence: Synthetic oligonucleotide"
ttggaggcaaggcatctctg

SEQ ID NO: 123 - DNA, 20 bp, Artificial Sequence
  source: /note="Description of Artificial Sequence: Synthetic oligonucleotide"
aggactcctgctgagaggag

SEQ ID NO: 124 - DNA, 20 bp, Artificial Sequence
  source: /note="Description of Artificial Sequence: Synthetic oligonucleotide"
ggagaactaaagggcgtgct

SEQ ID NO: 125 - DNA, 20 bp, Artificial Sequence
  source: /note="Description of Artificial Sequence: Synthetic oligonucleotide"
accaccacatgttctgggtg

SEQ ID NO: 126 - DNA, 20 bp, Artificial Sequence
  source: /note="Description of Artificial Sequence: Synthetic oligonucleotide"
gcttcctcttccaggctctg

SEQ ID NO: 127 - DNA, 97 bp, Artificial Sequence
  source: /note="Description of Artificial Sequence: Synthetic oligonucleotide"
  source: /note="Description of Combined DNA/RNA Molecule: Synthetic oligonucleotide"
ggggccactagggacaggauguuuuagagcuagaaauagcaaguuaaaauaaggcuaguccguuaucaacuugaaaaaguggcaccgagucggugcu

SEQ ID NO: 128 - DNA, 97 bp, Artificial Sequence; identical to SEQ ID NO: 127
  source: /note="Description of Artificial Sequence: Synthetic oligonucleotide"
  source: /note="Description of Combined DNA/RNA Molecule: Synthetic oligonucleotide"

SEQ ID NO: 129 - DNA, 103 bp, Artificial Sequence
  source: /note="Description of Artificial Sequence: Synthetic polynucleotide"
  source: /note="Description of Combined DNA/RNA Molecule: Synthetic polynucleotide"
ggggccactagggacaggauguuuuagagctgctgaaaagcauagcaaguuaaaauaaggcuaguccguuaucaacuugaaaaaguggcaccgagucggugcu

SEQ ID NO: 130 - DNA, 105 bp, Artificial Sequence
  source: /note="Description of Artificial Sequence: Synthetic polynucleotide"
  source: /note="Description of Combined DNA/RNA Molecule: Synthetic polynucleotide"
ggggccactagggacaggauguuuuagagctatgctgaaaagcatagcaaguuaaaauaaggcuaguccguuaucaacuugaaaaaguggcaccgagucggugcu

SEQ ID NO: 131 - DNA, 105 bp, Artificial Sequence
  source: /note="Description of Artificial Sequence: Synthetic polynucleotide"
  source: /note="Description of Combined DNA/RNA Molecule: Synthetic polynucleotide"
ggggccactagggacaggauguuuuagagctatgctgaaaagcatagcaaguuaaaauaaggcuaguccguuaucaacuugaaaaaguggcaccgagucggtgcu

SEQ ID NO: 132 - DNA, 105 bp, Artificial Sequence; identical to SEQ ID NO: 131
  source: /note="Description of Artificial Sequence: Synthetic polynucleotide"
  source: /note="Description of Combined DNA/RNA Molecule: Synthetic polynucleotide"

SEQ ID NO: 133 - DNA, 36 bp, Artificial Sequence
  source: /note="Description of Artificial Sequence: Synthetic oligonucleotide"
tacttccaatccaatgcaccccgttctcctgtggat

SEQ ID NO: 134 - DNA, 40 bp, Artificial Sequence
  source: /note="Description of Artificial Sequence: Synthetic oligonucleotide"
ttatccacttccaatgttattactccctcccaggatcctc

SEQ ID NO: 135 - DNA, 39 bp, Artificial Sequence
  source: /note="Description of Artificial Sequence: Synthetic oligonucleotide"
  source: /note="Description of Combined DNA/RNA Molecule: Synthetic oligonucleotide"
gccactagggacaggatgucucagagctatgctgtcctg

SEQ ID NO: 136 - DNA, 39 bp, Artificial Sequence
  source: /note="Description of Artificial Sequence: Synthetic oligonucleotide"
  source: /note="Description of Combined DNA/RNA Molecule: Synthetic oligonucleotide"
gccactagggacaggaugucucagagctatgctgtcctg

SEQ ID NO: 137 - DNA, 39 bp, Artificial Sequence; identical to SEQ ID NO: 135
  source: /note="Description of Artificial Sequence: Synthetic oligonucleotide"
  source: /note="Description of Combined DNA/RNA Molecule: Synthetic oligonucleotide"

SEQ ID NO: 138 - DNA, 56 bp, Artificial Sequence
  source: /note="Description of Artificial Sequence: Synthetic oligonucleotide"
  source: /note="Description of Combined DNA/RNA Molecule: Synthetic oligonucleotide"
  modified_base (1)..(15): a, c, t, g, unknown or other
  modified_base (16)..(20): a, c, u, g, unknown or other
nnnnnnnnnnnnnnnnnnnnguuuuaguactctgtaattttaggtatgaggtagac

SEQ ID NO: 139 - DNA, 56 bp, Artificial Sequence; identical to SEQ ID NO: 138
  source: /note="Description of Artificial Sequence: Synthetic oligonucleotide"
  source: /note="Description of Combined DNA/RNA Molecule: Synthetic oligonucleotide"
  modified_base (1)..(20): a, c, t, g, unknown or other

SEQ ID NO: 140 - DNA, 56 bp, Artificial Sequence
  source: /note="Description of Artificial Sequence: Synthetic oligonucleotide"
  source: /note="Description of Combined DNA/RNA Molecule: Synthetic oligonucleotide"
  modified_base (1)..(20): a, c, t, g, unknown or other
nnnnnnnnnnnnnnnnnnnnguuuuaguacucugtaattttaggtatgaggtagac

SEQ ID NO: 141 - DNA, 56 bp, Artificial Sequence
  source: /note="Description of Artificial Sequence: Synthetic oligonucleotide"
  source: /note="Description of Combined DNA/RNA Molecule: Synthetic oligonucleotide"
  modified_base (1)..(2): a, c, t, g, unknown or other
  modified_base (3)..(4): a, c, u, g, unknown or other
  modified_base (5)..(14): a, c, t, g, unknown or other
  modified_base (15)..(17): a, c, u, g, unknown or other
  modified_base (18)..(18): a, c, t, g, unknown or other
  modified_base (19)..(19): a, c, u, g, unknown or other
  modified_base (20)..(20): a, c, t, g, unknown or other
nnnnnnnnnnnnnnnnnnnnguuuuagtactctgtaattttaggtatgaggtagac

SEQ ID NO: 142 - RNA, 85 nt, Artificial Sequence
  source: /note="Description of Artificial Sequence: Synthetic oligonucleotide"
auuguacuuauaccuaaaauuacagaaucuacuaaaacaaggcaaaaugccguguuuaucucgucaacuuguuggcgagauuuuu

SEQ ID NO: 143 - DNA, 106 bp, Artificial Sequence
  source: /note="Description of Artificial Sequence: Synthetic polynucleotide"
  source: /note="Description of Combined DNA/RNA Molecule: Synthetic polynucleotide"
  modified_base (1)..(15): a, c, t, g, unknown or other
  modified_base (16)..(20): a, c, u, g, unknown or other
nnnnnnnnnnnnnnnnnnnnguuuuaguactctggaaacagaaucuacuaaaaacaaggccaaaaugccgguguuuaucuucgucaacuuuguuggcgaggauuuu

SEQ ID NO: 144 - DNA, 106 bp, Artificial Sequence; identical to SEQ ID NO: 143
  source: /note="Description of Artificial Sequence: Synthetic polynucleotide"
  source: /note="Description of Combined DNA/RNA Molecule: Synthetic polynucleotide"
  modified_base (1)..(20): a, c, t, g, unknown or other

SEQ ID NO: 145 - DNA, 106 bp, Artificial Sequence
  source: /note="Description of Artificial Sequence: Synthetic polynucleotide"
  source: /note="Description of Combined DNA/RNA Molecule: Synthetic polynucleotide"
  modified_base (1)..(20): a, c, t, g, unknown or other
nnnnnnnnnnnnnnnnnnnnguuuuaguacucuggaaacagaaucuacuaaaaacaaggccaaaaugccgguguuuaucuucgucaacuuuguuggcgaggauuuu

SEQ ID NO: 146 - DNA, 106 bp, Artificial Sequence
  source: /note="Description of Artificial Sequence: Synthetic polynucleotide"
  source: /note="Description of Combined DNA/RNA Molecule: Synthetic polynucleotide"
  modified_base (1)..(2): a, c, t, g, unknown or other
  modified_base (3)..(4): a, c, u, g, unknown or other
  modified_base (5)..(14): a, c, t, g, unknown or other
  modified_base (15)..(17): a, c, u, g, unknown or other
  modified_base (18)..(18): a, c, t, g, unknown or other
  modified_base (19)..(19): a, c, u, g, unknown or other
  modified_base (20)..(20): a, c, t, g, unknown or other
nnnnnnnnnnnnnnnnnnnnguuuuagtactctggaaacagaaucuacuaaaaacaaggccaaaaugccgguguuuaucuucgucaacuuuguuggcgaggauuuu

SEQ ID NO: 147 - DNA, 56 bp, Artificial Sequence
  source: /note="Description of Artificial Sequence: Synthetic oligonucleotide"
  source: /note="Description of Combined DNA/RNA Molecule: Synthetic oligonucleotide"
  modified_base (1)..(15): a, c, t, g, unknown or other
  modified_base (16)..(20): a, c, u, g, unknown or other
nnnnnnnnnnnnnnnnnnnnguuuuuguactctcaagatttaagtaactgtacaac

SEQ ID NO: 148 - DNA, 56 bp, Artificial Sequence
  source: /note="Description of Artificial Sequence: Synthetic oligonucleotide"
  source: /note="Description of Combined DNA/RNA Molecule: Synthetic oligonucleotide"
  modified_base (1)..(20): a, c, t, g, unknown or other
nnnnnnnnnnnnnnnnnnnnguuuuugtactctcaagatttaagtaactgtacaac

SEQ ID NO: 149 - DNA, 56 bp, Artificial Sequence
  source: /note="Description of Artificial Sequence: Synthetic oligonucleotide"
  source: /note="Description of Combined DNA/RNA Molecule: Synthetic oligonucleotide"
  modified_base (1)..(20): a, c, t, g, unknown or other
nnnnnnnnnnnnnnnnnnnnguuuuuguacuctcaagatttaagtaactgtacaac

SEQ ID NO: 150 - RNA, 89 nt, Artificial Sequence
  source: /note="Description of Artificial Sequence: Synthetic oligonucleotide"
cuuacacaguuacuuaaaucuugcagaagcuacaaagauaaggcuucaugccgaaaucaacacccugucauuuuauggcaggguguuuu

SEQ ID NO: 151 - DNA, 106 bp, Artificial Sequence
  source: /note="Description of Artificial Sequence: Synthetic polynucleotide"
  source: /note="Description of Combined DNA/RNA Molecule: Synthetic polynucleotide"
  modified_base (1)..(15): a, c, t, g, unknown or other
  modified_base (16)..(20): a, c, u, g, unknown or other
nnnnnnnnnnnnnnnnnnnnguuuuuguactcgaaagaagcuacaaagauuaaggcuucaaugccgaaauucaacacccuugucauuuuaauggcaggguuguuuu

SEQ ID NO: 152 - DNA, 106 bp, Artificial Sequence; identical to SEQ ID NO: 151
  source: /note="Description of Artificial Sequence: Synthetic polynucleotide"
  source: /note="Description of Combined DNA/RNA Molecule: Synthetic polynucleotide"
  modified_base (1)..(20): a, c, t, g, unknown or other

SEQ ID NO: 153 - DNA, 106 bp, Artificial Sequence
  source: /note="Description of Artificial Sequence: Synthetic polynucleotide"
  source: /note="Description of Combined DNA/RNA Molecule: Synthetic polynucleotide"
  modified_base (1)..(20): a, c, t, g, unknown or other
nnnnnnnnnnnnnnnnnnnnguuuuuguacucgaaagaagcuacaaagauuaaggcuucaaugccgaaauucaacacccuugucauuuuaauggcaggguuguuuu

SEQ ID NO: 154 - DNA, 56 bp, Artificial Sequence
  source: /note="Description of Artificial Sequence: Synthetic oligonucleotide"
  source: /note="Description of Combined DNA/RNA Molecule: Synthetic oligonucleotide"
  modified_base (1)..(15): a, c, t, g, unknown or other
  modified_base (16)..(20): a, c, u, g, unknown or other
nnnnnnnnnnnnnnnnnnnnguuguagcucccattctcatttcgcagtgctacaat

SEQ ID NO: 155 - DNA, 56 bp, Artificial Sequence
  source: /note="Description of Artificial Sequence: Synthetic oligonucleotide"
  source: /note="Description of Combined DNA/RNA Molecule: Synthetic oligonucleotide"
  modified_base (1)..(20): a, c, t, g, unknown or other
nnnnnnnnnnnnnnnnnnnnguuguagctcccattctcatttcgcagtgctacaat

SEQ ID NO: 156 - DNA, 56 bp, Artificial Sequence; identical to SEQ ID NO: 154
  source: /note="Description of Artificial Sequence: Synthetic oligonucleotide"
  source: /note="Description of Combined DNA/RNA Molecule: Synthetic oligonucleotide"
  modified_base (1)..(20): a, c, t, g, unknown or other

SEQ ID NO: 157 - RNA, 119 nt, Artificial Sequence
  source: /note="Description of Artificial Sequence: Synthetic polynucleotide"
auugucgcacugcgaaaugagaaccguugcuacaauaaggccgucugaaaagaugugccgcaacgcucugccccuuaaagcuucugcuuuaaggggcaucguuuauuucgguuaaaaau

SEQ ID NO: 158 - DNA, 110 bp, Artificial Sequence
  source: /note="Description of Artificial Sequence: Synthetic polynucleotide"
  source: /note="Description of Combined DNA/RNA Molecule: Synthetic polynucleotide"
  modified_base (1)..(15): a, c, t, g, unknown or other
  modified_base (16)..(20): a, c, u, g, unknown or other
nnnnnnnnnnnnnnnnnnnnguuguagcucccattctcgaaagagaaccgguugcuacaaauaaggccguucugaaaagaaugugccgcaaacgcucugcccccuuaaag

SEQ ID NO: 159 - DNA, 110 bp, Artificial Sequence; identical to SEQ ID NO: 158
  source: /note="Description of Artificial Sequence: Synthetic polynucleotide"
  source: /note="Description of Combined DNA/RNA Molecule: Synthetic polynucleotide"
  modified_base (1)..(20): a, c, t, g, unknown or other

SEQ ID NO: 160 - DNA, 110 bp, Artificial Sequence; identical to SEQ ID NO: 158
  source: /note="Description of Artificial Sequence: Synthetic polynucleotide"
  source: /note="Description of Combined DNA/RNA Molecule: Synthetic polynucleotide"
  modified_base (1)..(20): a, c, t, g, unknown or other

SEQ ID NO: 161 - DNA, 56 bp, Artificial Sequence
  source: /note="Description of Artificial Sequence: Synthetic oligonucleotide"
  source: /note="Description of Combined DNA/RNA Molecule: Synthetic oligonucleotide"
  modified_base (1)..(14): a, c, t, g, unknown or other
  modified_base (15)..(20): a, c, u, g, unknown or other
nnnnnnnnnnnnnnnnnnnnguuuuuguactctcaagatttaagtaaccgtaaaac

SEQ ID NO: 162 - DNA, 56 bp, Artificial Sequence
  source: /note="Description of Artificial Sequence: Synthetic oligonucleotide"
  source: /note="Description of Combined DNA/RNA Molecule: Synthetic oligonucleotide"
  modified_base (1)..(20): a, c, t, g, unknown or other
nnnnnnnnnnnnnnnnnnnnguuuuugtactctcaagatttaagtaaccgtaaaac

SEQ ID NO: 163 - DNA, 56 bp, Artificial Sequence
  source: /note="Description of Artificial Sequence: Synthetic oligonucleotide"
  source: /note="Description of Combined DNA/RNA Molecule: Synthetic oligonucleotide"
  modified_base (1)..(20): a, c, t, g, unknown or other
nnnnnnnnnnnnnnnnnnnnguuuuuguacucucaagatttaagtaaccgtaaaac

SEQ ID NO: 164 - RNA, 90 nt, Artificial Sequence
  source: /note="Description of Artificial Sequence: Synthetic oligonucleotide"
cuugcacgguuacuuaaaucuugcugagccuacaaagauaaggcuuuaugccgaauucaagcaccccauguuuugacaugaggugcuuuu

SEQ ID NO: 165 - DNA, 106 bp, Artificial Sequence
  source: /note="Description of Artificial Sequence: Synthetic polynucleotide"
  source: /note="Description of Combined DNA/RNA Molecule: Synthetic polynucleotide"
  modified_base (1)..(15): a, c, t, g, unknown or other
  modified_base (16)..(20): a, c, u, g, unknown or other
nnnnnnnnnnnnnnnnnnnnguuuuuguactcgaaagagccuacaaagauuaaggcuuuaaugccgaauuucaagcacccccauguuuuggacaugagguugcuuu

SEQ ID NO: 166 - DNA, 106 bp, Artificial Sequence; identical to SEQ ID NO: 165
  source: /note="Description of Artificial Sequence: Synthetic polynucleotide"
  source: /note="Description of Combined DNA/RNA Molecule: Synthetic polynucleotide"
  modified_base (1)..(20): a, c, t, g, unknown or other

SEQ ID NO: 167 - DNA, 106 bp, Artificial Sequence; identical to SEQ ID NO: 165
  source: /note="Description of Artificial Sequence: Synthetic polynucleotide"
  source: /note="Description of Combined DNA/RNA Molecule: Synthetic polynucleotide"
  modified_base (1)..(20): a, c, t, g, unknown or other

SEQ ID NO: 168 - RNA, 11 nt, Artificial Sequence
  source: /note="Description of Artificial Sequence: Synthetic oligonucleotide"
aauuucuacug

SEQ ID NO: 169 - DNA, 11 bp, Artificial Sequence
  source: /note="Description of Artificial Sequence: Synthetic oligonucleotide"
  source: /note="Description of Combined DNA/RNA Molecule: Synthetic oligonucleotide"
aauutctacug

SEQ ID NO: 170 - RNA, 11 nt, Artificial Sequence
  source: /note="Description of Artificial Sequence: Synthetic oligonucleotide"
aauuucuacug

SEQ ID NO: 171 - DNA, 11 bp, Artificial Sequence
  source: /note="Description of Artificial Sequence: Synthetic oligonucleotide"
  source: /note="Description of Combined DNA/RNA Molecule: Synthetic oligonucleotide"
aauutctacug

SEQ ID NO: 172 - RNA, 33 nt, Artificial Sequence
  source: /note="Description of Artificial Sequence: Synthetic oligonucleotide"
  modified_base (9)..(33): a, c, u, g, unknown or other
uuguagaunnnnnnnnnnnnnnnnnnnnnnnnn

SEQ ID NO: 173 - RNA, 33 nt, Artificial Sequence; identical to SEQ ID NO: 172
  source: /note="Description of Artificial Sequence: Synthetic oligonucleotide"
  modified_base (9)..(33): a, c, u, g, unknown or other

SEQ ID NO: 174 - RNA, 28 nt, Artificial Sequence
  source: /note="Description of Artificial Sequence: Synthetic oligonucleotide"
  modified_base (9)..(28): a, c, u, g, unknown or other
uuguagaunnnnnnnnnnnnnnnnnnnn

SEQ ID NO: 175 - RNA, 28 nt, Artificial Sequence
  source: /note="Description of Artificial Sequence: Synthetic oligonucleotide"
  modified_base (9)..(28): a, c, u, g, unknown or other
uuguagaunnnnnnnnnnnnnnnnnnnn

SEQ ID NO: 176 - DNA, 33 bp, Artificial Sequence
  source: /note="Description of Artificial Sequence: Synthetic oligonucleotide"
  source: /note="Description of Combined DNA/RNA Molecule: Synthetic oligonucleotide"
  modified_base (9)..(33): a, c, t, g, unknown or other
uuguagaunnnnnnnnnnnnnnnnnnnnnnnnn

SEQ ID NO: 177 - DNA, 33 bp, Artificial Sequence; identical to SEQ ID NO: 176
  source: /note="Description of Artificial Sequence: Synthetic oligonucleotide"
  source: /note="Description of Combined DNA/RNA Molecule: Synthetic oligonucleotide"
  modified_base (9)..(10): a, c, u, g, unknown or other
  modified_base (11)..(33): a, c, t, g, unknown or other

SEQ ID NO: 178 - DNA, 33 bp, Artificial Sequence; identical to SEQ ID NO: 176
  source: /note="Description of Artificial Sequence: Synthetic oligonucleotide"
  source: /note="Description of Combined DNA/RNA Molecule: Synthetic oligonucleotide"
  modified_base (9)..(13): a, c, u, g, unknown or other
  modified_base (14)..(33): a, c, t, g, unknown or other

SEQ ID NO: 179 - DNA, 33 bp, Artificial Sequence; identical to SEQ ID NO: 176
  source: /note="Description of Artificial Sequence: Synthetic oligonucleotide"
  source: /note="Description of Combined DNA/RNA Molecule: Synthetic oligonucleotide"
  modified_base (9)..(18): a, c, u, g, unknown or other
  modified_base (19)..(33): a, c, t, g, unknown or other

SEQ ID NO: 180 - DNA, 33 bp, Artificial Sequence
  source: /note="Description of Artificial Sequence: Synthetic oligonucleotide"
  source: /note="Description of Combined DNA/RNA Molecule: Synthetic oligonucleotide"
  modified_base (9)..(33): a, c, u, g, unknown or other
uugtagaunnnnnnnnnnnnnnnnnnnnnnnnn

SEQ ID NO: 181 - DNA, 33 bp, Artificial Sequence; identical to SEQ ID NO: 180
  source: /note="Description of Artificial Sequence: Synthetic oligonucleotide"
  source: /note="Description of Combined DNA/RNA Molecule: Synthetic oligonucleotide"
  modified_base (9)..(33): a, c, u, g, unknown or other

SEQ ID NO: 182 - DNA, 28 bp, Artificial Sequence
  source: /note="Description of Artificial Sequence: Synthetic oligonucleotide"
  source: /note="Description of Combined DNA/RNA Molecule: Synthetic oligonucleotide"
  modified_base (9)..(28): a, c, u, g, unknown or other
uugtagaunnnnnnnnnnnnnnnnnnnn

SEQ ID NO: 183 - DNA, 28 bp, Artificial Sequence
  source: /note="Description of Artificial Sequence: Synthetic oligonucleotide"
  source: /note="Description of Combined DNA/RNA Molecule: Synthetic oligonucleotide"
  modified_base (9)..(28): a, c, u, g, unknown or other
uuguagaunnnnnnnnnnnnnnnnnnnn

SEQ ID NO: 184 - DNA, 33 bp, Artificial Sequence; identical to SEQ ID NO: 180
  source: /note="Description of Artificial Sequence: Synthetic oligonucleotide"
  source: /note="Description of Combined DNA/RNA Molecule: Synthetic oligonucleotide"
  modified_base (9)..(33): a, c, t, g, unknown or other

SEQ ID NO: 185 - DNA, 33 bp, Artificial Sequence; identical to SEQ ID NO: 180
  source: /note="Description of Artificial Sequence: Synthetic oligonucleotide"
  source: /note="Description of Combined DNA/RNA Molecule: Synthetic oligonucleotide"
  modified_base (9)..(10): a, c, u, g, unknown or other
  modified_base (11)..(33): a, c, t, g, unknown or other

SEQ ID NO: 186 - DNA, 33 bp, Artificial Sequence; identical to SEQ ID NO: 180
  source: /note="Description of Artificial Sequence: Synthetic oligonucleotide"
  source: /note="Description of Combined DNA/RNA Molecule: Synthetic oligonucleotide"
  modified_base (9)..(13): a, c, u, g, unknown or other
  modified_base (14)..(33): a, c, t, g, unknown or other

SEQ ID NO: 187 - DNA, 33 bp, Artificial Sequence; identical to SEQ ID NO: 180
  source: /note="Description of Artificial Sequence: Synthetic oligonucleotide"
  source: /note="Description of Combined DNA/RNA Molecule: Synthetic oligonucleotide"
  modified_base (9)..(18): a, c, u, g, unknown or other
  modified_base (19)..(33): a, c, t, g, unknown or other

SEQ ID NO: 188 - DNA, 44 bp, Artificial Sequence
  source: /note="Description of Artificial Sequence: Synthetic oligonucleotide"
  source: /note="Description of Combined DNA/RNA Molecule: Synthetic oligonucleotide"
  modified_base (20)..(44): a, c, u, g, unknown or other
aauuucuacuguugtagaunnnnnnnnnnnnnnnnnnnnnnnnn

SEQ ID NO: 189 - DNA, 44 bp, Artificial Sequence
  source: /note="Description of Artificial Sequence: Synthetic oligonucleotide"
  source: /note="Description of Combined DNA/RNA Molecule: Synthetic oligonucleotide"
  modified_base (20)..(44): a, c, u, g, unknown or other
aauutctacuguuguagaunnnnnnnnnnnnnnnnnnnnnnnnn

SEQ ID NO: 190 - DNA, 44 bp, Artificial Sequence
  source: /note="Description of Artificial Sequence: Synthetic oligonucleotide"
  source: /note="Description of Combined DNA/RNA Molecule: Synthetic oligonucleotide"
  modified_base (20)..(44): a, c, u, g, unknown or other
aauutctacuguugtagaunnnnnnnnnnnnnnnnnnnnnnnnn

SEQ ID NO: 191 - DNA, 44 bp, Artificial Sequence
  source: /note="Description of Artificial Sequence: Synthetic oligonucleotide"
  source: /note="Description of Combined DNA/RNA Molecule: Synthetic oligonucleotide"
  modified_base (20)..(44): a, c, t, g, unknown or other
aauuucuacuguuguagaunnnnnnnnnnnnnnnnnnnnnnnnn

SEQ ID NO: 192 - DNA, 44 bp, Artificial Sequence; identical to SEQ ID NO: 189
  source: /note="Description of Artificial Sequence: Synthetic oligonucleotide"
  source: /note="Description of Combined DNA/RNA Molecule: Synthetic oligonucleotide"
  modified_base (20)..(44): a, c, t, g, unknown or other

SEQ ID NO: 193 - DNA, 44 bp, Artificial Sequence; identical to SEQ ID NO: 189
  source: /note="Description of Artificial Sequence: Synthetic oligonucleotide"
  source: /note="Description of Combined DNA/RNA Molecule: Synthetic oligonucleotide"
  modified_base (20)..(21): a, c, u, g, unknown or other
  modified_base (22)..(44): a, c, t, g, unknown or other

SEQ ID NO: 194 - DNA, 44 bp, Artificial Sequence; identical to SEQ ID NO: 189
  source: /note="Description of Artificial Sequence: Synthetic oligonucleotide"
  source: /note="Description of Combined DNA/RNA Molecule: Synthetic oligonucleotide"
  modified_base (20)..(24): a, c, u, g, unknown or other
  modified_base (25)..(44): a, c, t, g, unknown or other

SEQ ID NO: 195 - DNA, 44 bp, Artificial Sequence; identical to SEQ ID NO: 189
  source: /note="Description of Artificial Sequence: Synthetic oligonucleotide"
  source: /note="Description of Combined DNA/RNA Molecule: Synthetic oligonucleotide"
  modified_base (20)..(29): a, c, u, g, unknown or other
  modified_base (30)..(44): a, c, t, g, unknown or other

SEQ ID NO: 196 - DNA, 44 bp, Artificial Sequence; identical to SEQ ID NO: 188
  source: /note="Description of Artificial Sequence: Synthetic oligonucleotide"
  source: /note="Description of Combined DNA/RNA Molecule: Synthetic oligonucleotide"
  modified_base (20)..(44): a, c, t, g, unknown or other

SEQ ID NO: 197 - DNA, 44 bp, Artificial Sequence; identical to SEQ ID NO: 188
  source: /note="Description of Artificial Sequence: Synthetic oligonucleotide"
  source: /note="Description of Combined DNA/RNA Molecule: Synthetic oligonucleotide"
  modified_base (20)..(21): a, c, u, g, unknown or other
  modified_base (22)..(44): a, c, t, g, unknown or other

SEQ ID NO: 198 - DNA, 44 bp, Artificial Sequence; identical to SEQ ID NO: 188
  source: /note="Description of Artificial Sequence: Synthetic oligonucleotide"
  source: /note="Description of Combined DNA/RNA Molecule: Synthetic oligonucleotide"
  modified_base (20)..(24): a, c, u, g, unknown or other
  modified_base (25)..(44): a, c, t, g, unknown or other

SEQ ID NO: 199 - DNA, 44 bp, Artificial Sequence; identical to SEQ ID NO: 188
  source: /note="Description of Artificial Sequence: Synthetic oligonucleotide"
  source: /note="Description of Combined DNA/RNA Molecule: Synthetic oligonucleotide"
  modified_base (20)..(29): a, c, u, g, unknown or other
  modified_base (30)..(44): a, c, t, g, unknown or other

SEQ ID NO: 200 - DNA, 44 bp, Artificial Sequence; identical to SEQ ID NO: 190
  source: /note="Description of Artificial Sequence: Synthetic oligonucleotide"
  source: /note="Description of Combined DNA/RNA Molecule: Synthetic oligonucleotide"
  modified_base (20)..(44): a, c, t, g, unknown or other

SEQ ID NO: 201 - DNA, 44 bp, Artificial Sequence; identical to SEQ ID NO: 190
  source: /note="Description of Artificial Sequence: Synthetic oligonucleotide"
  source: /note="Description of Combined DNA/RNA Molecule: Synthetic oligonucleotide"
  modified_base (20)..(21): a, c, u, g, unknown or other
  modified_base (22)..(44): a, c, t, g, unknown or other

SEQ ID NO: 202 - DNA, 44 bp, Artificial Sequence; identical to SEQ ID NO: 190
  source: /note="Description of Artificial Sequence: Synthetic oligonucleotide"
  source: /note="Description of Combined DNA/RNA Molecule: Synthetic oligonucleotide"
  modified_base (20)..(24): a, c, u, g, unknown or other
  modified_base (25)..(44): a, c, t, g, unknown or other

SEQ ID NO: 203 - DNA, 44 bp, Artificial Sequence; identical to SEQ ID NO: 190
  source: /note="Description of Artificial Sequence: Synthetic oligonucleotide"
  source: /note="Description of Combined DNA/RNA Molecule: Synthetic oligonucleotide"
  modified_base (20)..(29): a, c, u, g, unknown or other
  modified_base (30)..(44): a, c, t, g, unknown or other

SEQ ID NO: 204 - DNA, 97 bp, Artificial Sequence
  source: /note="Description of Artificial Sequence: Synthetic polynucleotide"
  source: /note="Description of Combined DNA/RNA Molecule: Synthetic polynucleotide"
tacgcgtacgcgtacgugugguuuuagagcuagaaauagcaaguuaaaauaaggcuaguccguuaucaacuugaaaaaguggcaccgagucggugcu

SEQ ID NO: 205 - DNA, 105 bp, Artificial Sequence
  source: /note="Description of Artificial Sequence: Synthetic polynucleotide"
  source: /note="Description of Combined DNA/RNA Molecule: Synthetic polynucleotide"
tacgcgtacgcgtacgugugguuuuagagctatgctgaaaagcatagcaaguuaaaauaaggcuaguccguuaucaacuugaaaaaguggcaccgagucggugcu

SEQ ID NO: 206 - DNA, 105 bp, Artificial Sequence
  source: /note="Description of Artificial Sequence: Synthetic polynucleotide"
  source: /note="Description of Combined DNA/RNA Molecule: Synthetic polynucleotide"
tacgcgtacgcgtacgugugguuuuagagctatgctgaaaagcatagcaaguuaaaauaaggcuaguccguuaucaacuugaaaaaguggcaccgagucggtgcu

SEQ ID NO: 207 - RNA, 98 nt, Artificial Sequence
  source: /note="Description of Artificial Sequence: Synthetic oligonucleotide"
ggcguacgcguacgugugguuuuagagcuagaaauagcaaguuaaaauaaggcuaguccguuaucaacuugaaaaaguggcaccgagucggugcuuuu

SEQ ID NO: 208 - DNA, 60 bp, Artificial Sequence
  source: /note="Description of Artificial Sequence: Synthetic oligonucleotide"
ctacactctttccctacacgacgctcttccgatctaaggcgcaaatgagtagcagcgcac

SEQ ID NO: 209 - DNA, 57 bp, Artificial Sequence
  source: /note="Description of Artificial Sequence: Synthetic oligonucleotide"
caagcagaagacggcatacgagctcttccgatctcacctgctgggaattgtaccgta

SEQ ID NO: 210 - DNA, 60 bp, Artificial Sequence
  source: /note="Description of Artificial Sequence: Synthetic oligonucleotide"
ctacactctttccctacacgacgctcttccgatctggaacgcaaatgagtagcagcgcac

SEQ ID NO: 211 - DNA, 60 bp, Artificial Sequence
  source: /note="Description of Artificial Sequence: Synthetic oligonucleotide"
ctacactctttccctacacgacgctcttccgatctccttcgcaaatgagtagcagcgcac

SEQ ID NO: 212 - DNA, 60 bp, Artificial Sequence
  source: /note="Description of Artificial Sequence: Synthetic oligonucleotide"
ctacactctttccctacacgacgctcttccgatctgaagcgcaaatgagtagcagcgcac

SEQ ID NO: 213 - DNA, 60 bp, Artificial Sequence
  source: /note="Description of Artificial Sequence: Synthetic oligonucleotide"
ctacactctttccctacacgacgctcttccgatctaggacgcaaatgagtagcagcgcac

SEQ ID NO: 214 - DNA, 43 bp, Artificial Sequence
  source: /note="Description of Artificial Sequence: Synthetic oligonucleotide"
aatgatacggcgaccaccgagatctacactctttccctacacg

SEQ ID NO: 215 - DNA, 18 bp, Artificial Sequence
  source: /note="Description of Artificial Sequence: Synthetic oligonucleotide"
caagcagaagacggcata

SEQ ID NO: 216 - DNA, 56 bp, Zea mays
cagcgcacgtatatatacgcgtacgcgtacgtgtgaggtatatatatcctccgccg

SEQ ID NO: 217 - DNA, 55 bp, Zea mays
cagcgcacgtatatatacgcgtacgcgtacgttgaggtatatatatcctccgccg

SEQ ID NO: 218 - DNA, 57 bp, Zea mays
cagcgcacgtatatatacgcgtacgcgtacgttgtgaggtatatatatcctccgccg

SEQ ID NO: 219 - DNA, 55 bp, Zea mays
cagcgcacgtatatatacgcgtacgcgtacggtgaggtatatatatcctccgccg

SEQ ID NO: 220 - DNA, 27 bp, Zea mays
cagcgcacgtatatatatcctccgccg

SEQ ID NO: 221 - DNA, 55 bp, Zea mays; identical to SEQ ID NO: 217

SEQ ID NO: 222 - DNA, 52 bp, Zea mays
cagcgcacgtatatatacgcgtacgcgtatgaggtatatatatcctccgccg

SEQ ID NO: 223 - DNA, 55 bp, Zea mays; identical to SEQ ID NO: 217

SEQ ID NO: 224 - DNA, 97 bp, Artificial Sequence
  source: /note="Description of Artificial Sequence: Synthetic oligonucleotide"
  source: /note="Description of Combined DNA/RNA Molecule: Synthetic oligonucleotide"
ggccgaggtcgactaccggcguuuuagagcuagaaauagcaaguuaaaauaaggcuaguccguuaucaacuugaaaaaguggcaccgagucggugcu

SEQ ID NO: 225 - DNA, 105 bp, Artificial Sequence
  source: /note="Description of Artificial Sequence: Synthetic polynucleotide"
  source: /note="Description of Combined DNA/RNA Molecule: Synthetic polynucleotide"
ggccgaggtcgactaccggcguuuuagagctatgctgaaaagcatagcaaguuaaaauaaggcuaguccguuaucaacuugaaaaaguggcaccgagucggugcu

SEQ ID NO: 226 - DNA, 105 bp, Artificial Sequence
  source: /note="Description of Artificial Sequence: Synthetic polynucleotide"
  source: /note="Description of Combined DNA/RNA Molecule: Synthetic polynucleotide"
ggccgaggtcgactaccggcguuuuagagctatgctgaaaagcatagcaaguuaaaauaaggcuaguccguuaucaacuugaaaaaguggcaccgagucggtgcu

SEQ ID NO: 227 - RNA, 124 nt, Artificial Sequence
  source: /note="Description of Artificial Sequence: Synthetic polynucleotide"
gggccgaggucgacuaccggcguuuuagagcuaugcuguuuuggaaacaaaacagcauagcaaguuaaaauaaggcuaguccguuaucaacuugaaaaaguggcaccgagucggugcuuuuuuu

SEQ ID NO: 228 - DNA, 54 bp, Artificial Sequence
  source: /note="Description of Artificial Sequence: Synthetic oligonucleotide"
caagcagaagacggcatacgagctcttccgatctgccggctggcattgtctctg

SEQ ID NO: 229 - DNA, 58 bp, Artificial Sequence
  source: /note="Description of Artificial Sequence: Synthetic oligonucleotide"
ctacactctttccctacacgacgctcttccgatctttccggacccgttcggcctcagt

SEQ ID NO: 230 - DNA, 58 bp, Artificial Sequence
  source: /note="Description of Artificial Sequence: Synthetic oligonucleotide"
ctacactctttccctacacgacgctcttccgatctggaaggacccgttcggcctcagt

SEQ ID NO: 231 - DNA, 58 bp, Artificial Sequence
  source: /note="Description of Artificial Sequence: Synthetic oligonucleotide"
ctacactctttccctacacgacgctcttccgatctccttggacccgttcggcctcagt

SEQ ID NO: 232 - DNA, 58 bp, Artificial Sequence
  source: /note="Description of Artificial Sequence: Synthetic oligonucleotide"
ctacactctttccctacacgacgctcttccgatcttcctggacccgttcggcctcagt

SEQ ID NO: 233 - DNA, 58 bp, Artificial Sequence
  source: /note="Description of Artificial Sequence: Synthetic oligonucleotide"
ctacactctttccctacacgacgctcttccgatctaaggggacccgttcggcctcagt

SEQ ID NO: 234 - DNA, 39 bp, Zea mays
agtccgctggccgaggtcgactaccggccggtgaagcac

SEQ ID NO: 235 - DNA, 40 bp, Zea mays
agtccgctggccgaggtcgactaccaggccggtgaagcac

SEQ ID NO: 236 - DNA, 40 bp, Zea mays
agtccgctggccgaggtcgacttgccggccggtgaagcac

SEQ ID NO: 237 - DNA, 22 bp, Zea mays
agtccgctggccggtgaagcac

SEQ ID NO: 238 - DNA, 37 bp, Zea mays
agtccgctggccgaggtcgaccaggccggtgaagcac

SEQ ID NO: 239 - DNA, 40 bp, Zea mays
agtccgctggccgaggtcgactacctggccggtgaagcac

SEQ ID NO: 240 - DNA, 18 bp, Zea mays
agtccgccagtgaagcac

SEQ ID NO: 241 - DNA, 38 bp, Zea mays
agtccgctggccgaggtcgactacggccggtgaagcac

SEQ ID NO: 242 - DNA, 40 bp, Zea mays
agtccgctggccgaggtcgactacccggccggtgaagcac

SEQ ID NO: 243 - DNA, 40 bp, Zea mays; identical to SEQ ID NO: 235

SEQ ID NO: 244 - DNA, 22 bp, Zea mays
agtccgctggccggtgaagcac

SEQ ID NO: 245 - DNA, 38 bp, Zea mays; identical to SEQ ID NO: 241

SEQ ID NO: 246 - DNA, 37 bp, Zea mays
agtccgctggccgaggtcgacttggccggtgaagcac

SEQ ID NO: 247 - DNA, 40 bp, Zea mays; identical to SEQ ID NO: 235

SEQ ID NO: 248 - DNA, 38 bp, Zea mays; identical to SEQ ID NO: 241

SEQ ID NO: 249 - DNA, 40 bp, Zea mays; identical to SEQ ID NO: 239

SEQ ID NO: 250 - DNA, 40 bp, Zea mays; identical to SEQ ID NO: 242

SEQ ID NO: 251 - DNA, 28 bp, Zea mays
agtccgctggtcaaggccggcgaagcac

SEQ ID NO: 252 - DNA, 22 bp, Zea mays
agtccgctggccggtgaagcac

SEQ ID NO: 253 - DNA, 37 bp, Zea mays
agtccgctggccgaggtcgactaagccggtgaagcac

SEQ ID NO: 254 - DNA, 24 bp, Zea mays
agtccgctggccgaggtgaagcac